European Patent Specification EP 3 512 567 B1, published November 1, 2023. Title: Cardiac Regeneration Using Cardiomyocyte-Specific Modified RNA. Applicant: Icahn School of Medicine at Mount Sinai Zangi, Lior. The sequence listing filed with the application follows.

SEQUENCE LISTING (10 sequences)

SEQ ID NO: 1 - DNA, 536 bp, Artificial Sequence
  synthetic oligonucleotide
ttggaccctcgtacagaagctaatacgactcactatagggaaataagagagaaaagaagagtaagaagaaatataagagccaccatgtacgtgagatttgaggttcctgaggacatgcagaacgaagctctgagtctgctggagaaggttagggagagcggtaaggtaaagaaaggtaccaacgagacgacaaaggctgtggagaggggactggcaaagctcgtttacatcgcagaggatgttgacccgcctgagatcgttgctcatctgcccctcctctgcgaggagaagaatgtgccgtacatttacgttaaaagcaagaacgaccttggaagggctgtgggcattgaggtgccatgcgcttcggcagcgataatcaacgagggagagctgagaaaggagcttggaagccttgtggagaagattaaaggccttcagaagtaagctgccttctgcggggcttgccttctggccatgcccttcttctctcccttgcacctgtacctcttggtctttgaataaagcctgagtaggaa

SEQ ID NO: 2 - DNA, 620 bp, Artificial Sequence
  synthetic oligonucleotide
ttggaccctcgtacagaagctaatacgactcactatagggaaataagagagaaaagaagagtaagaagaaatataagagccaccatgtacgtgagatttgaggttcctgaggacatgcagaacgaagctctgagtctgctggagaaggttagggagagcggtaaggtaaagaaaggtaccaacgagacgacaaaggctgtggagaggggactggcaaagctcgtttacatcgcagaggatgttgacccgcctgagatcgttgctcatctgcccctcctctgcgaggagaagaatgtgccgtacatttacgttaaaagcaagaacgaccttggaagggctgtgggcattgaggtgccatgcgcttcggcagcgataatcaacgagggagagctgagaaaggagcttggaagccttgtggagaagattaaaggccttcagaagtaatacatacttctttacattccatacatacttctttacattccatacatacttctttacattccatacatacttctttacattccagctgccttctgcggggcttgccttctggccatgcccttcttctctcccttgcacctgtacctcttggtctttgaataaagcctgagtaggaa

SEQ ID NO: 3 - DNA, 624 bp, Artificial Sequence
  synthetic oligonucleotide
ttggaccctcgtacagaagctaatacgactcactatagggaaataagagagaaaagaagagtaagaagaaatataagagccaccatgtacgtgagatttgaggttcctgaggacatgcagaacgaagctctgagtctgctggagaaggttagggagagcggtaaggtaaagaaaggtaccaacgagacgacaaaggctgtggagaggggactggcaaagctcgtttacatcgcagaggatgttgacccgcctgagatcgttgctcatctgcccctcctctgcgaggagaagaatgtgccgtacatttacgttaaaagcaagaacgaccttggaagggctgtgggcattgaggtgccatgcgcttcggcagcgataatcaacgagggagagctgagaaaggagcttggaagccttgtggagaagattaaaggccttcagaagtaaacaagctttttgctcgtcttatacaagctttttgctcgtcttatacaagctttttgctcgtcttatacaagctttttgctcgtcttatgctgccttctgcggggcttgccttctggccatgcccttcttctctcccttgcacctgtacctcttggtctttgaataaagcctgagtaggaa

SEQ ID NO: 4 - DNA, 708 bp, Artificial Sequence
  synthetic oligonucleotide
ttggaccctcgtacagaagctaatacgactcactatagggaaataagagagaaaagaagagtaagaagaaatataagagccaccatgtacgtgagatttgaggttcctgaggacatgcagaacgaagctctgagtctgctggagaaggttagggagagcggtaaggtaaagaaaggtaccaacgagacgacaaaggctgtggagaggggactggcaaagctcgtttacatcgcagaggatgttgacccgcctgagatcgttgctcatctgcccctcctctgcgaggagaagaatgtgccgtacatttacgttaaaagcaagaacgaccttggaagggctgtgggcattgaggtgccatgcgcttcggcagcgataatcaacgagggagagctgagaaaggagcttggaagccttgtggagaagattaaaggccttcagaagtaatacatacttctttacattccatacatacttctttacattccatacatacttctttacattccatacatacttctttacattccaacaagctttttgctcgtcttatacaagctttttgctcgtcttatacaagctttttgctcgtcttatacaagctttttgctcgtcttatgctgccttctgcggggcttgccttctggccatgcccttcttctctcccttgcacctgtacctcttggtctttgaataaagcctgagtaggaa

SEQ ID NO: 5 - DNA, 832 bp, Artificial Sequence
  synthetic oligonucleotide
ttggaccctcgtacagaagctaatacgactcactatagggaaaggtgggcgtgatccgaaaggtgacccggatctggggcgtgatccgaaaggtgacccggaaagccaccatgggctcggtgtccaaccagcagtttgcaggtggctgcgccaaggcagcggagaaggcgccagaggaggcgccgcctgacgcggcccgagcggcagacgagccgcagctgctgcacggggccggcatctgtaagtggttcaacgtgcgcatggggttcggcttcctgtctatgaccgcccgcgctggggtcgcgctcgaccccccggtggacgtctttgtgcaccagagcaagctgcacatggaagggttccgaagcctcaaggagggtgaggcggtggagttcacctttaagaagtctgccaagggtctggaatccatccgtgtcactggccctggtggtgtgttctgtattgggagtgagcggcggccaaaagggaagaacatgcagaagcgaagatccaaaggagacaggtgctacaactgcggtgggctagaccatcatgccaaggaatgcaagctgccaccccagcccaagaagtgccacttttgccaaagcatcaaccatatggtggcctcgtgtccactgaaggcccagcagggccccagttctcagggaaagcctgcctacttccgggaggaagaggaagagatccacagccctgccctgctcccagaagcccagaattgagctgccttctgcggggcttgccttctggccatgcccttcttctctcccttgcacctgtacctcttggtctttgaataaagcctgagtaggaa

SEQ ID NO: 6 - DNA, 1798 bp, Artificial Sequence
  synthetic oligonucleotide
ttggaccctcgtacagaagctaatacgactcactatagggaaaggtgggcgtgatccgaaaggtgacccggatctggggcgtgatccgaaaggtgacccggaaagccaccatgccgaagccacacagtgaagcagggactgccttcattcagacccagcagctccatgcagccatggctgacaccttcctggaacacatgtgccgcctggacattgactctgcccccatcacggcccgcaacactggcatcatttgtaccattgggcctgcttcccgatctgtggagatgctgaaggagatgattaagtctggaatgaatgtggctcggctgaatttctctcatggaacccatgagtaccatgcagagaccatcaagaatgtccgtgaagccacagaaagctttgcatctgatcccattctctaccgtcctgttgcggtggctctggatacaaagggacctgagatccggactggactcatcaagggcagcggcaccgctgaggtggagctgaagaagggagccactctgaagatcaccctggacaacgcttacatggagaagtgtgacgagaacatcctgtggctggactacaagaacatctgcaaggtggtggaggtgggcagcaagatctacgtggacgatgggctcatctcactgcaggtgaaggagaaaggcgctgacttcctggtgacggaggtggagaatggtggctccttgggcagcaagaagggcgtgaacctgccgggcgctgctgtggatctccccgctgtgtcggaaaaggacatccaggacctgaagtttggggtggagcaggatgtggacatggtgtttgcatctttcatccgcaaggcagccgacgtgcatgaagtcaggaaggtgctgggagagaagggcaagaacatcaagatcatcagcaaaatcgagaaccatgaaggcgtccgcaggtttgatgagatcttggaggccagtgatgggatcatggtggctcgtggtgacctgggcattgagattcctgcagagaaggtcttcctggctcagaagatgatgatcgggcgatgcaaccgagctgggaagcctgtcatctgtgccacacagatgctggagagcatgatcaagaagccacgccccacccgtgctgaaggcagtgatgtggccaatgcagtcctggatggagcagactgcatcatgctgtctggagaaacagccaagggggactaccctctggaggctgttcgcatgcagcacctgattgcccgagaggcagaggctgccatctaccacttgcagctattcgaggaactccgccgcctggcgcccattaccagcgaccccacagaagctgccgccgtgggtgccgtggaggcctccttcaagtgctgcagtggggccattatcgtgctcaccaagtctggcaggagtgctcaccaagtggccaggtaccgccctcgggctcctatcattgccgtgactcgaaatccccagactgctcgccaggcccatctgtaccgtggcatcttccctgtgctgtgtaaggatgccgtgctgaatgcctgggctgaggatgtcgaccttcgtgtaaacttggccatggatgttggcaaggcccgaggcttcttcaagaagggagatgtggtcattgtgctgaccgggtggcgccctggctctggattcaccaacaccatgcgtgtagtgcctgtaccttgagctgccttctgcggggcttgccttctggccatgcccttcttctctcccttgcacctgtacctcttggtctttgaataaagcctgagtaggaa

SEQ ID NO: 7 - DNA, 975 bp, Artificial Sequence
  synthetic oligonucleotide
ttggaccctcgtacagaagctaatacgactcactatagggaaaggtgggcgtgatccgaaaggtgacccggatctggggcgtgatccgaaaggtgacccggaaagccaccatggtgagcaagggcgaggagctgttcaccggggtggtgcccatcctggtcgagctggacggcgacgtaaacggccacaagttcagcgtgtccggcgagggcgagggcgatgccacctacggcaagctgaccctgaagttcatctgcaccaccggcaagctgcccgtgccctggcccaccctcgtgaccaccctgacctacggcgtgcagtgcttcagccgctaccccgaccacatgaagcagcacgacttcttcaagtccgccatgcccgaaggctacgtccaggagcgcaccatcttcttcaaggacgacggcaactacaagacccgcgccgaggtgaagttcgagggcgacaccctggtgaaccgcatcgagctgaagggcatcgacttcaaggaggacggcaacatcctggggcacaagctggagtacaactacaacagccacaacgtctatatcatggccgacaagcagaagaacggcatcaaggtgaacttcaagatccgccacaacatcgaggacggcagcgtgcagctcgccgaccactaccagcagaacacccccatcggcgacggccccgtgctgctgcccgacaaccactacctgagcacccagtccgccctgagcaaagaccccaacgagaagcgcgatcacatggtcctgctggagttcgtgaccgccgccgggatcactctcggcatggacgagctgtacaagggagatccaaaaaagaagagaaaggtaggcgatccaaaaaagaagagaaaggtaggtgatccaaaaaagaagagaaaggtataagctgccttctgcggggcttgccttctggccatgcccttcttctctcccttgcacctgtacctct

SEQ ID NO: 8 - DNA, 1021 bp, Artificial Sequence
  synthetic oligonucleotide
ttggaccctcgtacagaagctaatacgactcactatagggaaaggtgggcgtgatccgaaaggtgacccggatctggggcgtgatccgaaaggtgacccggaaagccaccatggattcatacctgctgatgtggggactgctcacgttcatcatggtgcctggctgccaggcagagctctgtgacgatgacccgccagagatcccacacgccacattcaaagccatggcctacaaggaaggaaccatgttgaactgtgaatgcaagagaggtttccgcagaataaaaagcgggtcactctatatgctctgtacaggaaactctagccactcgtcctgggacaaccaatgtcaatgcacaagctctgccactcggaacacaacgaaacaagtgacacctcaacctgaagaacagaaagaaaggaaaaccacagaaatgcaaagtccaatgcagccagtggaccaagcgagccttccaggtcactgcagggaacctccaccatgggaaaatgaagccacagagagaatttatcatttcgtggtggggcagatggtttattatcagtgcgtccagggatacagggctctacacagaggtcctgctgagagcgtctgcaaaatgacccacgggaagacaaggtggacccagccccagctcatatgcacaggtgaaatggagaccagtcagtttccaggtgaagagaagcctcaggcaagccccgaaggccgtcctgagagtgagacttcctgcctcgtcacaacaacagattttcaaatacagacagaaatggctgcaaccatggagacgtccatatttacaacagatctccaggtagcagtggccggctgtgttttcctgctgatcagcgtcctcctcctgagtgggctcacctggcagcggagacagaggaagagtagaagaacaatctaggctgccttctgcggggcttgccttctggccatgcccttcttctctcccttgcacctgtacctcttggtctttgaataaagcctgagtaggaa

SEQ ID NO: 9 - DNA, 27 bp, Artificial Sequence
  synthetic oligonucleotide
ttggaccctcgtacagaagctaatacg

SEQ ID NO: 10 - DNA, 150 bp, Artificial Sequence
  synthetic oligonucleotide
tttttttttttttttttttttttttttttttttttttttttttttttttttttttttttttttttttttttttttttttttttttttttttttttttttttttttttttttttttttttttcttcctactcaggctttattcaaagacca